European Patent Specification EP 3 704 220 B1, published April 15, 2026. Title: MEDICAL CLEANING COMPOSITIONS AND USES THEREOF. Applicant: Novozymes A/S. The sequence listing filed with the application follows.

SEQUENCE LISTING (24 sequences)

SEQ ID NO: 1 - protein, 324 aa, Terribacillus saccharophilus
QDQEKGITIDISRKYYSIKTLKAIVDEISANGGDYLQLHFSDNESYAIASEFLGQNSENPNSAYLTKKELLSLIAYSNDRNIMVIPDIDLPAHSKGWLNIMKEKDSGLYTDIVTDYSEDTLDYHNNAVALYTANQLLDEVLDLFYQPKFAGKQRIVLGGDEVPGSGAHQTDFIRFMNQIAKTAKASNYEPQMWNDSITPEGIQNLDRSFSILYWKQSTLSNGAQSLDVQDFEENGLSVYNYNAYSLYFLPSTRFTQEDITEQIDYMKWAYAYNKFFYISDYYKQVDTPNVKGSSLVFWGEHANDLSQEGLLKQEKPLIQNFLGL

SEQ ID NO: 2 - protein, 324 aa, Terribacillus goriensis
QDQEKGITIDISRKYYSIETLKSIIDEISANGGDYLQLHFSDNERYAIASEFLGQNGENPNSTYLTKKELLSLIAYSNDRDIMVIPDIDLPAHSRGWLNIMKEKDSGLYTDIVTDYSEDTLDYHNNAVALYTANQLLDEVLDLFYQPKFAGKQRIVLGGDEVPGSGVHQTDFIRFMNQIAETAKASNYKPQMWNDSITPEGIQNLDRSFSILYWKQSTLSNGAQGLDVQDFEENGLSVYNYNAYSLYFLPATRFTQEDITEQIDYMKWAYAYNKFFYISDYYKQVDTSNVKGSSLVFWGEHANDLSQEGLLKQEKPLIQNFLGL

SEQ ID NO: 3 - protein, 324 aa, Terribacillus saccharophilus
KDQEKGITIDISRKYYSIGTLKAIVDEINANGGDYLQLHFSDNESYAIASEFLGQNSENPNSTYLTKKELLSLIAYSNDRNIMVIPDIDLPAHSKGWLNVMKEKDSGLYTDIVTDYSEDTLDYHNNAAALYTANQLLDEVLDLFYQPKFAGKQRIVLGGDEVPGSGAHQTDFIRFMNQIDETAKASNYEPQMWNDSITPEGIQNLDRSFSILYWKQSTLSSGAQGLDVQNFEEKGFSVYNYNAYSLYFLPSTRFTQEDITEQIDYMKWAYAYNKFFYISDYYKQVDTSNVKGSSLVFWGEHANDLSQEGLLEQEKPLIQNFLSL

SEQ ID NO: 4 - protein, 324 aa, Terribacillus saccharophilus [sequence omitted]

SEQ ID NO: 5 - protein, 324 aa, Terribacillus saccharophilus
KDQEKGISIDISRKYYSIGTLKAIIDEISANGGDYLQLHFSDNESYAIASDYLGQISDTPNNTYLTKNDLLSLIAYSNDRNILIIPDMDLPAHSRGWLELMKVKDRELYTDIVTDYSNETLDYHNNTDALNTANQLLNEILELFYQPKFAGKQRIVLGGDEVPGSEIHQLDFIRFINQIASTAKASNYAPQMWNDSITAEGIQNLDKSFSILYWKQSTLSNGAQSLEVQDFEDWDFPVYNYNAYSLYFLPSIRFTDEDITEQMNYMKWAYAYNKFFYISDYYKSVDASNVKGSSLTFWGEHATDLSQEELLEQELPLIKKFLSL

SEQ ID NO: 6 - protein, 461 aa, Curtobacterium oceanosedimentum
ADRNTSAAEAAVTSIAPRATITGVAAISAATSSRTTVRTTLTLENRSGERESAADAWLYLAGGGARYALGHAPVRALAAGARATVRTTLRVPSRAPAGKYAVLACAGPYSKQACRTSGTTVTVGTAARARPETGVMLDVARAYYPVSLIEQYVDLLAEHGGGFLHLHLTDDQNVGIESAVLGQTPANAVLRNGVYTSRVTGRPFLSAAQARAISAYAAKRGIAIVPEVDSPGHMAAAFALLEARHGATWVDRIRSGESELDTSVPESATLAAELLREVTQTFPSSRTVHIGGDEWGADVSADERVGWMNAMAAAIGDREVWAWNDGIDRASVGRLDPRIHVTYWSFDGDTEDAAERRERRARRASATDLQRAGIDLLNYNSYYLYEVPTDLDPADSEYTVADLREHWSLRAWDGDSGARLAAPMSGAAVAIWGEDLDGAPSEALLRWSAPHVTAMIETAAS

SEQ ID NO: 7 - protein, 445 aa, Curtobacterium flaccumfaciens
DTAVSAVTVTKVTASTTGTVVRTTLKVENTAPVRKPASSVWLYLSAGTEKYTLGRVAVKALAAGSSTSVTAVRGTPSRAAAGKYSVLACAGAYSAKQCRTSTATVTTKPTKRARPETGVMLDVARAYYPVALIKRYIDLLADDGGRFLHLHLTDDQNVGIESTVLGQTPANADLDHGVYTSRVTHRPFLSAAQARTISAYGAERGVAIVPEIDTPGHMAAAFALLEAQHGTKWVDRIRSGENELDTSAPESLALAKKLYAEVQRTFPSSRTVHIGGDEWGDDVTAAQRVTWMNAMAAALDDREVWAWNDGIDRVAVGRLDPRIHVTYWSFDGDTEDAAERRERRARRASAVDLQQAGIDQLNYNSYYLYEVPTDLDPADSDYTVADLRENWSLRAWDGDSGSLLAAPMSGAAVAIWGEDLEDPPSDALLRWSAPHVTAMIETAAS

SEQ ID NO: 8 - protein, 445 aa, Curtobacterium luteum
DTAVSAVTVTKVTASTTGTAVRTTLKVENTAPVRKPASSVWLYLSAGTEKYTLGRVAVKALSAGSSTSVTAVRGTPSRAAAGKYWVLACAGAYSAKQCRTSTATVTTKPTKRARPETGVMLDVARAYYPVALIKRYIDLLADDGGRFLHLHLTDDQNVGIESTVLGQTPANADLDHGVYTSRVTHRPFLSAAQARTISEYGAERGVTIVPEIDTPGHMAAAFALLEAQHGTKWVDRIRSGENELDTSAPESLVLAKKLYAEVQRTFPSSRTVHIGGDEWGDDVTAAHRVAWMNEMAATLGNREVWAWNDGIDRVAVGRLDPRIHVTYWSFDGDTEDAAERRERRARRASAVDLQQAGIDQLNYNSYYLYEVPTDLDPADSDYTVADLRENWSLRAWDGDSGSLLAAPMSGAAVAIWGEDLEDPPSDALLRWSAPHVTAMIETAAS

SEQ ID NO: 9 - protein, 458 aa, Curtobacterium oceanosedimentum
IGGSAGTADASGAPRLVVTKVTASSTTTSTRTTVRTTLTVKNTSVARKPAADAWLSLTAGSKRYTLGHVSVQSLAAGASATIHATHTAPPRAPAGKYAVLACTGAFSLSKCGTSATTVTTARATRARPDTGVMLDVARAYYPVALIEQYIALLADHGGRFLHLHLTDDQNVGIESEVLGQTLANADLRDGVYTSRITGRPFLSAAQAREISRYAAQRGIAIIPEIDTPGHMAAAFALLEAGHGKQWVDRIRSGESELDTSAPGSSALAARLLQEVTRTFPSSRTVHIGGDEWGDDVTADERVQWLNTMAAAVGNRAVWAWNDGIDRAAIGRLDPRIHVTYWSFDGDTEDATERRERRERRAGANDLYAAGIDLLNYNSYYLYEVPTDLDAADSEYTVADLRENWSLRTWDGDSGARLAGPTSGAAVAIWGEDLEAPPSDALLRWSAPHVLAMIETAGS

SEQ ID NO: 10 - protein, 450 aa, Curtobacterium Leaf154
AGSTTSTVTVTQVTATTTASSTGTAVRTTLKIKNTAAVRKPASSAWLYLSAGTKKYTLGRVAVKALAAGSSTSVTAVRGTPSRATAGEYSVLACAGAYSAKQCRTSTATVTTKPTKRARPETGVMLDVARAYYPVALIKRYIDLLADDGGRFLHLHLTDDQNVGIESTVLGQTLANADLDEGVYTSRVTRRPFLSAAQARTISDYAARRGVAIVPEIDTPGHMTAAFDLLEAQHGTKWVDRIRSGENELDTSTPGSLALAKKLYAEVQRTFPASRTVHIGGDEWGDDVSAAERVAWMNAMAAALGNREVWAWNDGIDRVAVGRLDPRIHVTYWSFDGDTEDAAERRERRARRASAVDLQQAGIDMLNYNSYYLYEVPTDLDPADSEYTVADLRENWSLRTWDGDSGSLLAAPMSGAAVAIWGEDLEDPPSDALLRWSAPHVTAMIETAAS

SEQ ID NO: 11 - protein, 359 aa, Aggregatibacter actinomycetemcomitans
CVKGNSIHPQKTSTKQTGLMLDIARHFYSPEVIKSFIDTISLSGGNFLHLHFSDHENYAIESHLLNQRAENAVQGKDGIYINPYTGKPFLSYRQLDDIKAYAKAKGIELIPELDSPNHMTAIFKLVQKDRGIKYLQGLKSRQVDDEIDITNADSIAFMQSLMSEVIDIFGDTSQHFHIGGDEFGYSVESNHEFITYANKLSYFLEKKGLKTRMWNDGLIKSTFEQINPNIEITYWSYDGDTQDKNEAAERRDMRVSLPELLAKGFTVLNYNSYYLYIVPKASPTFSQDAAFAAKDVIKNWDLGVWDGRNTKNRVQNTHEIAGAALSIWGEDAKALKDETIQKNTKSLLEAVIHKANGDE

SEQ ID NO: 12 - protein, 346 aa, Haemophilus sputorum
QNSTKQSGLMLDISRRFYSVETIKQFIDDIAQANGTFLHLHFADHENYALESTFLNQRAENAIVQNGIYINPKTNKPFLTYEQIDQIIRYAQEKQIELIPEVDSPAHIKGILTLLRLEKGEDYVNQIALNQDELNLDSPESLTMMKTLVDEVCYIFGYSAQHFHIGGDEFNYASNFIRYVNALNQHINQKGLITRMWNDGLLQQNIDELDKNIEITYWSFDGDAQEKNDIVERRATRISLPTLLDKGFKALNYNSYYLYFIPKDNGNIATDAKFALNDLKQNWQLLRWDGNYETQPIQQAENLIGAAFSIWGEHAGKLSDDVIHQATSPLIQATIIQTNAKTTGPN

SEQ ID NO: 13 - protein, 352 aa, Actinobacillus suis
MNHSQIKEAGLTLDIARRFYPVETIKQFIDTIHHAGGTFLHLHFSDHENYALESTYLDQSEANAIVKDGTYYNPKTNKPFLTYKQIHDIIYYAKSKNIELVPEVDTPNHMTAIFRLLEAKHGKDYVKKLKSKMNDEEIDITNPESIEVIKTLIAEVIYIFGHASEHFHIGGDEFGYSVETNHEFISYVNTLNQFINEKGKITRIWNDGLIKNNLNQLNKNVEITYWSYDGDAQESQDIAERRKIRANLPELLENGFKVLNYNSYYLYFVPKGNANITHDSKYATEDVLNNWKLGLWDGQNKENMVENTKNIIGSSLSIWGERSGSLSSEVIEESTQDLLKAVIQKTNDPKSH

SEQ ID NO: 14 - protein, 352 aa, Actinobacillus capsulatus DSM 19761
MNHSQIKEAGLTLDIARRFYPVETIKQFIDTIHHAGGTFLHLHFSDHENYALESTYLDQLEANAIVKDGTYYNPTTNKPFLTYKQINDIIYYAKSKNIELVPEVDTPNHMTAIFRLLEAKHSKDYVKRLKSKMNDEEIDITNLESIEVIKTLIAEVIYIFGHASEHFHIGGDEFGYSVETNHEFITYVNTLNQFINNKGKITRIWNDGLIKNNLNQLNKNVEITYWSYDGDAQESQDIAERRKIRVNLPELLENGFKVLNYNSYYLYFVPKGNANITHDSKHATEDVLKNWKLGLWDGQNKENIVENTKNIIGSSLSIWGEHSGSLSSAVIEESTQELLKAVIQKTNDPKSH

SEQ ID NO: 15 - protein, 352 aa, Actinobacillus equuli subsp. equuli
MNHSQIKEAGLTLDIARRFYPVETIKQFIDTIHHAGGTFLHLHFSDHENYALESSYLDQSEENAIVKDGTYYNPKTNKPFLTYKQIDDIIYYAKSKNIELVPEVDTPNHMTAIFNLLEIKHGEAYVKNLKSKMNDEEIDITNPESIEVIKTLIAEVIYIFGHASEHFHIGGDEFGYSVETNHEFISYVNTLNQFINEKGKITRIWNDGLIKNNLNQLNKNVEITYWSYDGDAQKSQDIAERRKIRADLPELLENGFKVLNYNSYYLYFVPKGNANITHDSKYATEDVLNNWKLGLWDGKNKENEVKNTKNIIGSSLSIWGERSGSLSSEVIEESTQDLLKAVIQKTNDPKSH

SEQ ID NO: 16 - protein, 359 aa, Aggregatibacter actinomycetemcomitans
CVKGNSIYPQKISTKQTGLMLDIARHFYSPEVIKSFIDTISLSGGNFLHLHFSDHENYAIESHLLNQRAENAVQGKDGIYINPYTGKPFLSYRQLDDIKAYAKAKGIELIPELDSPNHMTAIFKLVQKDRGVKYLQGLKSRQVDDEIDITNADSIAFMQSLMNEVIDIFGDTSQHFHIGGDEFGYSVESNHEFITYANKLSYFLEKKGLKTRMWNDGLIKSTFEQINPNIEITYWSYDGDTQDKNEAAERRDMRVSLPELLAKGFTVLNYNSYYLYIVPKASPTFSQDAAFAAKDVIKNWDLGVWDGRNTKNRVQNTHEIAGAALSIWGEDAKALKDETIQKNTKSLLEAVIHKTNGDE

SEQ ID NO: 17 - protein, 359 aa, Aggregatibacter actinomycetemcomitans
CVKGNSIYPQKTSTKQTGLMLDIARHFYSPEVIKSFIDTISLSGGNFLHLHFSDHENYAIESHLLNQRAENAVQGKDGIYINPYTGKPFLSYRQLDDIKAYAKAKGIELIPELDSPNHMTAIFKLVQKDRGVKYLQGLKSRQVDDEIDITNADSITFMQSLMSEVIDIFGDTSQHFHIGGDEFGYSVESNHEFITYANKLSYFLEKKGLKTRMWNDGLIKNTFEQINPNIEITYWSYDGDTQDKNEAAERRDMRVSLPELLAKGFTVLNYNSYYLYIVPKASPTFSQDAAFAAKDVIKNWDLGVWDGRNTKNRVQNTHEIAGAALSIWGEDAKALKDETIQKNTKSLLEAVIHKTNGDE

SEQ ID NO: 18 - protein, 351 aa, Actinobacillus pleuropneumoniae
MDLPKKESGLTLDIARRFYTVDTIKQFIDTIHQAGGTFLHLHFSDHENYALESSYLEQREENATEKNGTYFNPKTNKPFLTYKQLNEIIYYAKERNIEIVPEVDSPNHMTAIFDLLTLKHGKEYVKGLKSPYIAEEIDINNPEAVEVIKTLIGEVIYIFGHSSRHFHIGGDEFSYAVENNHEFIRYVNTLNDFINSKGLITRVWNDGLIKNNLSELNKNIEITYWSYDGDAQAKEDIQYRREIRADLPELLANGFKVLNYNSYYLYFVPKSGSNIHNDGKYAAEDVLNNWTLGKWDGKNSSNHVQNTQNIIGSSLSIWGERSSALNEQTIQQASKNLLKAVIQKTNDPKSH

SEQ ID NO: 19 - protein, 331 aa, Lactobacillus paraplantarum
NSSTLNTSQGVMLDLGRHPLDETAIKAVISAAAEQHMQYVELHLSDNEHLCFQSAYLGNAASATVLSATTLEQLVAYANQLNIELVPDVDLPSHAGAILRQLQQTHPDIYNTVKLDDETIDYTKPAAISLATTLYGELDASFNNQSQHDLMLGADEVPGSASAYIELTTFINQVSRFQNQHGFNTSIWNDSLLKNELTRLDSNITINYWSQSGNNTDVAIIADRYANRVSVPDILASGHPIVNCNSYATYYQIKNIGNVNDDDYFINYLNHTFRPNIFNEIDTNGHNQDWTIEDGVTTNGILVSLWGADSEHVTPTAIVNFIKRMTIPRSF

SEQ ID NO: 20 - protein, 353 aa, Lactobacillus apinorum
TLADTSNDTKRIGLSLDCSRTYYSPSTIKKYIDLLKKDHGTYLQLHLNDNERYGVESSTLGQTTQNATLKDGVYYNNKTHLAFLSKNQLLDVIQYGYTHGIEVIPEIDLPGHAQSIFKLLSYTSEGKKLVKELENKDGYNEMYYNKQATIDFSKKLLSEYVGMLPSGYHIIVGADEITISDKSDQEAVVKYINAIDDYVNANHLKLEMWNDSFHKAVLSKYHKDILINYWSLTGEVSSSKDRKDNIRMRATLPELNKAGFKTINYNSYYLYMITDPTSFTNESKKIWTSEFKKWKMNMWNDESTKDITKSANNIGAAISIWGEYPNQYTGDQTYNKTYYYVDTFLKAQDKFTK

SEQ ID NO: 21 - protein, 331 aa, Lactobacillus paraplantarum
NSSTLNTSQGVMLDLGRHPLDETAIKAVISAAAEQHMQYVELHLSDNEHLCFQSAYLGNAASATVLSATTLEQLVAYANQLNIELVPDVDLPSHAGAILRQLQQTHPDIYNTVKLDDETIDYTKPAAVSLATTLYGELDASFNNQSQHDLMLGADEVSGSASAYIELTTFINQVSRFQNQNGFNTSIWNDSLLKNELNRLDSNITINYWSQSGNNTDAAIIADRYANRASVPDILASGHPIVNCNSYATYYQFKNIGNVNDDNYFINYLNHTFRPNIFNEIDTNGHNQDWTIEDGVTTNGILVSLWGADSEHVTPTAIVNFIKRMAIPRSF

SEQ ID NO: 22 - protein, 482 aa, Streptococcus merionis
QEPIVKLSGGVMVDVARRYYSLNSLKSIIDTVSENKGDFVHLHLTDDQNYGLESQFLNQTASNAIYNQDDQSYTNPNTNRKFLSYGQLAELKSYAGSKGIRLIPEIDTPAHTGGLKALLPYAEPAVTSQFKWVSWDEDRQLDLDAATTQEAVRQLYMELVRELPGLEYIHIGGDEISGGLIQGQSFISHVNQLCDYLAGQGIKTQIWNDSLSRQLLPSLNRNVEIAYWGYLPHRNPDLATASDLSDQDFKLLNYNGYYLAFVPKPSEKLQSDALFAANDILKTWNLSQFHMDTGDSINSLKNVIGAAFSIWSEESAGLTDEEIFSAMGSPIRALLTVINQENIKRNENTTTTTTESMTEATTTITTEPTTQSTTESTTTTTTESTTETTTTVTTESTTKSTTEGTTETTTPIPPMPQPTTSPETSTATHATTTNPSTSKDGNKLSKSKRILPSTGETIGVLSVAGLALFLFVGLTYYRHKKN

SEQ ID NO: 23 - protein, 323 aa, Staphylococcus cohnii
QDFQKGINVDIARKDYSLKSLKKIVDTIHENNGDYLQLHFSDNENYAIESQFFKHENIASQNYLSQQELKNLIHYSNKLNIMVVPEFDLPSHSKAWLLLLKNENSNLHENIVSDYSDETIDFFSNQKALEISKRQIKEILNLFHQPNFQKEQRIVLGGDEVPGGKSYQNDFINFMNEIGEYAYQNGYEPQIWNDSITKNGLKLLKNYFSVIFWKQSNNENNEPGITVEDFLDYNFKVYNYNFYSLYFLPSKNYSPTDIEEQTSYISWAYNHNSFYYLKNPYYEVDSLNIQGSALSFWGEHATGMREEEVLNQELPLIRTYLNK

SEQ ID NO: 24 - protein, 321 aa, Staphylococcus fleurettii
ESIQEGVSVDIARKEYSLESLKQIVDTIHENNGQYLQLHFSDDENYAIESDYFSHQGIPNENYLTKAEIKSLIAYSNELNVMVVPDIDFPSHSKALLSLIKNEDKDLYNQIISDYSDNTFDFFSNDKALAISKRHIGEITTLFNQPKYNGQQRIVLGGDEVPGGGAYQSDFISYMNNIGSYAAGQGYEPQMWNDMISHEGIKSLNDTFSILYWKQNENSKSDLTVEDFAEYDFKIYNYNFYSLYFLPSNQFTNADIEEQADYISWAYAYNKFFYTNEPYQEVDSDNVKGSALSFWGEDALNMSQTELINQEIPLIKAYFSS